European Patent Specification EP 2 480 251 B1, published December 3, 2025. Title: CARRIER CONJUGATES OF IL-23-PEPTIDES AND THEIR INDUCED ANTIBODIES. Applicant: Zagury, Jean-François Ratsimandresy, Rojo. The sequence listing filed with the application follows.

SEQUENCE LISTING (141 sequences)

SEQ ID NO: 1 - protein, 19 aa, Homo Sapiens
LLPDSPVGQLHASLLGLSQ

SEQ ID NO: 2 - protein, 20 aa, Homo Sapiens
GSDIFTGEPSLLPDSPVGQL

SEQ ID NO: 3 - protein, 20 aa, Mus Musculus
DSDIFKGEPALLPDSPMEQL

SEQ ID NO: 4 - protein, 11 aa, Mus Musculus
KGEPALLPDSP

SEQ ID NO: 5 - protein, 11 aa, Homo Sapiens
TGEPSLLPDSP

SEQ ID NO: 6 - protein, 7 aa, Artificial
  sub-sequence of seq ID N°2 with C-terminal and N-terminal cystein
CTGEPSC

SEQ ID NO: 7 - protein, 8 aa, Artificial
  sub-sequence of seq ID N°2 with  N-terminal cystein and C-terminal cystein and tyrosin
CLPDSPCY

SEQ ID NO: 8 - protein, 15 aa, Artificial
  reverse sequence derived from SEQ ID N°2
VPSDPLLSPEGTFID

SEQ ID NO: 9 - protein, 11 aa, Artificial
  polypeptide
  MISC_FEATURE (1)..(1): T or K
  MISC_FEATURE (5)..(5): S or P or A
  MISC_FEATURE (7)..(7): L or F or H
  MISC_FEATURE (9)..(9): D or N
  MISC_FEATURE (10)..(10): S or G or D
  MISC_FEATURE (11)..(11): P or S
XGEPXLXPXXX

SEQ ID NO: 10 - protein, 11 aa, Canis lupus familiaris
TGEPSLLPDGP

SEQ ID NO: 11 - protein, 11 aa, Peromyscus maniculatus
TGEPSLLPDDP

SEQ ID NO: 12 - protein, 11 aa, Equus caballus
TGEPSLLPNGP

SEQ ID NO: 13 - protein, 20 aa, Artificial
  polypeptide
  MISC_FEATURE (1)..(1): G or D or A
  MISC_FEATURE (6)..(6): T or K
  MISC_FEATURE (10)..(10): S or P or A
  MISC_FEATURE (12)..(12): L or F or H
  MISC_FEATURE (14)..(14): D or N
  MISC_FEATURE (15)..(15): S or G or D
  MISC_FEATURE (16)..(16): P or S
  MISC_FEATURE (17)..(17): V or M
  MISC_FEATURE (18)..(18): G or S or E or D or A
XSDIFXGEPXLXPXXXXXQL

SEQ ID NO: 14 - protein, 20 aa, Canis lupus familiaris
GSDIFTGEPSLLPDGPVGQL

SEQ ID NO: 15 - protein, 20 aa, Rattus norvegicus
DSDIFTGEPSLLPDSPVDQL

SEQ ID NO: 16 - protein, 20 aa, Peromyscus maniculatus
DSDIFTGEPSLLPDDPVGQL

SEQ ID NO: 17 - protein, 20 aa, Onychomys leucogaster
DSDIFTGEPSLLPDGPVGQL

SEQ ID NO: 18 - protein, 20 aa, Cervus elaphus
GSDIFTGEPSLLPDGPVDQL

SEQ ID NO: 19 - protein, 20 aa, Equus caballus
GSDIFTGEPSLLPNGPVDQL

SEQ ID NO: 20 - protein, 20 aa, Bos taurus
GSDIFTGEPSLLPNGPVDQL

SEQ ID NO: 21 - protein, 20 aa, Sus scrofa
GSDIFTGEPSLHPDGSVGQL

SEQ ID NO: 22 - protein, 20 aa, Cavia porcellus
GSDIFTGEPPLFPDGPVSQL

SEQ ID NO: 23 - protein, 20 aa, Mus musculus
DSDIFKGEPALLPDSPMEQL

SEQ ID NO: 24 - protein, 20 aa, Homo Sapiens
GSDIFTGEPSLLPDSPVGQL

SEQ ID NO: 25 - protein, 11 aa, Artificial sequence
  IL-23p19 fragment
  misc_feature (1)..(1): Xaa can be G, D, or A
  misc_feature (6)..(6): Xaa can be T or K
  misc_feature (10)..(10): Xaa can be S, P, or A
XSDIFXGEPXL

SEQ ID NO: 26 - protein, 11 aa, Artificial sequence
  IL-23p19 fragment
  misc_feature (5)..(5): Xaa can be T or K
  misc_feature (9)..(9): Xaa can be S, P, or A
  misc_feature (11)..(11): Xaa can be L, H, or F
SDIFXGEPXLX

SEQ ID NO: 27 - protein, 11 aa, Artificial sequence
  IL23p19 fragment
  misc_feature (4)..(4): Xaa can be T or K
  misc_feature (8)..(8): Xaa can be S, P, or A
  misc_feature (10)..(10): Xaa can be L, H, or F
DIFXGEPXLXP

SEQ ID NO: 28 - protein, 11 aa, Artificial sequence
  IL-23p19 fragment
  misc_feature (3)..(3): Xaa can be T or K
  misc_feature (7)..(7): Xaa can be S, P, or A
  misc_feature (9)..(9): Xaa can be L, H, or F
  misc_feature (11)..(11): Xaa can be D or N
IFXGEPXLXPX

SEQ ID NO: 29 - protein, 11 aa, Artificial sequence
  IL-23p19 fragment
  misc_feature (2)..(2): Xaa can be T or K
  misc_feature (6)..(6): Xaa can be S, P, or A
  misc_feature (8)..(8): Xaa can be L, H, or F
  misc_feature (10)..(10): Xaa can be D or N
  misc_feature (11)..(11): Xaa can be G, S, or D
FXGEPXLXPXX

SEQ ID NO: 30 - protein, 11 aa, Artificial sequence
  IL-23p19 fragment
  misc_feature (1)..(1): Xaa can be T or K
  misc_feature (5)..(5): Xaa can be S, P, or A
  misc_feature (7)..(7): Xaa can be L, H, or F
  misc_feature (9)..(9): Xaa can be D or N
  misc_feature (10)..(10): Xaa can be G, S, or D
  misc_feature (11)..(11): Xaa can be P or S
XGEPXLXPXXX

SEQ ID NO: 31 - protein, 11 aa, Artificial sequence
  IL-23p19 fragment
  misc_feature (4)..(4): Xaa can be S, P, or A
  misc_feature (6)..(6): Xaa can be L, H, or F
  misc_feature (8)..(8): Xaa can be D or N
  misc_feature (9)..(9): Xaa can be G, S, or D
  misc_feature (10)..(10): Xaa can be P or S
  misc_feature (11)..(11): Xaa can be V or M
GEPXLXPXXXX

SEQ ID NO: 32 - protein, 11 aa, Artificial sequence
  IL-23p19 fragment
  misc_feature (3)..(3): Xaa can be S, P, or A
  misc_feature (5)..(5): Xaa can be L, H, or F
  misc_feature (7)..(7): Xaa can be D or N
  misc_feature (8)..(8): Xaa can be G, S, or D
  misc_feature (9)..(9): Xaa can be P or S
  misc_feature (10)..(10): Xaa can be V or M
  misc_feature (11)..(11): Xaa can be G, D, S, E, or A
EPXLXPXXXXX

SEQ ID NO: 33 - protein, 11 aa, Artificial sequence
  IL-23p19 fragment
  misc_feature (2)..(2): Xaa can be S, P, or A
  misc_feature (4)..(4): Xaa can be L, H, or F
  misc_feature (6)..(6): Xaa can be D or N
  misc_feature (7)..(7): Xaa can be G, S, or D
  misc_feature (8)..(8): Xaa can be P or S
  misc_feature (9)..(9): Xaa can be V or M
  misc_feature (10)..(10): Xaa can be G, D, S, E, or A
PXLXPXXXXXQ

SEQ ID NO: 34 - protein, 11 aa, Artificial sequence
  IL-23p19 fragment
  misc_feature (1)..(1): Xaa can be S, P, or A
  misc_feature (3)..(3): Xaa can be L, H, or F
  misc_feature (5)..(5): Xaa can be D or N
  misc_feature (6)..(6): Xaa can be G, S, or D
  misc_feature (7)..(7): Xaa can be P or S
  misc_feature (8)..(8): Xaa can be V or M
  misc_feature (9)..(9): Xaa can be G, D, S, E, or A
XLXPXXXXXQL

SEQ ID NO: 35 - protein, 12 aa, Artificial sequence
  IL-23p19 fragment
  misc_feature (1)..(1): Xaa can be G, D, or A
  misc_feature (6)..(6): Xaa can be T or K
  misc_feature (10)..(10): Xaa can be S, P, or A
  misc_feature (12)..(12): Xaa can be L, H, or F
XSDIFXGEPXLX

SEQ ID NO: 36 - protein, 12 aa, Artificial sequence
  IL-23p19 fragment
  misc_feature (5)..(5): Xaa can be T or K
  misc_feature (9)..(9): Xaa can be S, P, or A
  misc_feature (11)..(11): Xaa can be L, H, or F
SDIFXGEPXLXP

SEQ ID NO: 37 - protein, 12 aa, Artificial sequence
  IL-23p19 fragment
  misc_feature (4)..(4): Xaa can be T or K
  misc_feature (8)..(8): Xaa can be S, P, or A
  misc_feature (10)..(10): Xaa can be L, H, or F
  misc_feature (12)..(12): Xaa can be D or N
DIFXGEPXLXPX

SEQ ID NO: 38 - protein, 12 aa, Artificial sequence
  IL-23p19 fragment
  misc_feature (3)..(3): Xaa can be T or K
  misc_feature (7)..(7): Xaa can be S, P, or A
  misc_feature (9)..(9): Xaa can be L, H, or F
  misc_feature (11)..(11): Xaa can be D or N
  misc_feature (12)..(12): Xaa can be G, S, or D
IFXGEPXLXPXX

SEQ ID NO: 39 - protein, 12 aa, Artificial sequence
  IL-23p19 fragment
  misc_feature (2)..(2): Xaa can be T or K
  misc_feature (6)..(6): Xaa can be S, P, or A
  misc_feature (8)..(8): Xaa can be L, H, or F
  misc_feature (10)..(10): Xaa can be D or N
  misc_feature (11)..(11): Xaa can be G, S, or D
  misc_feature (12)..(12): Xaa can be P or S
FXGEPXLXPXXX

SEQ ID NO: 40 - protein, 12 aa, Artificial sequence
  IL-23p19 fragment
  misc_feature (1)..(1): Xaa can be T or K
  misc_feature (5)..(5): Xaa can be S, P, or A
  misc_feature (7)..(7): Xaa can be L, H, or F
  misc_feature (9)..(9): Xaa can be D or N
  misc_feature (10)..(10): Xaa can be G, S, or D
  misc_feature (11)..(11): Xaa can be P or S
  misc_feature (12)..(12): Xaa can be V or M
XGEPXLXPXXXX

SEQ ID NO: 41 - protein, 12 aa, Artificial sequence
  IL-23p19 fragment
  misc_feature (4)..(4): Xaa can be S, P, or A
  misc_feature (6)..(6): Xaa can be L, H, or F
  misc_feature (8)..(8): Xaa can be D or N
  misc_feature (9)..(9): Xaa can be G, S, or D
  misc_feature (10)..(10): Xaa can be P or S
  misc_feature (11)..(11): Xaa can be V or M
  misc_feature (12)..(12): Xaa can be G, D, S, E, or A
GEPXLXPXXXXX

SEQ ID NO: 42 - protein, 12 aa, Artificial sequence
  IL-23p19 fragment
  misc_feature (3)..(3): Xaa can be S, P, or A
  misc_feature (5)..(5): Xaa can be L, H, or F
  misc_feature (7)..(7): Xaa can be D or N
  misc_feature (8)..(8): Xaa can be G, S, or D
  misc_feature (9)..(9): Xaa can be P or S
  misc_feature (10)..(10): Xaa can be V or M
  misc_feature (11)..(11): Xaa can be G, D, S, E, or A
EPXLXPXXXXXQ

SEQ ID NO: 43 - protein, 12 aa, Artificial sequence
  IL-23p19 fragment
  misc_feature (2)..(2): Xaa can be S, P, or A
  misc_feature (4)..(4): Xaa can be L, H, or F
  misc_feature (6)..(6): Xaa can be D or N
  misc_feature (7)..(7): Xaa can be G, S, or D
  misc_feature (8)..(8): Xaa can be P or S
  misc_feature (9)..(9): Xaa can be V or M
  misc_feature (10)..(10): Xaa can be G, D, S, E, or A
PXLXPXXXXXQL

SEQ ID NO: 44 - protein, 13 aa, Artificial sequence
  IL-23p19 fragment
  misc_feature (1)..(1): Xaa can be G, D, or A
  misc_feature (6)..(6): Xaa can be T or K
  misc_feature (10)..(10): Xaa can be S, P, or A
  misc_feature (12)..(12): Xaa can be L, H, or F
XSDIFXGEPXLXP

SEQ ID NO: 45 - protein, 13 aa, Artificial sequence
  IL-23p19 fragment
  misc_feature (5)..(5): Xaa can be T or K
  misc_feature (9)..(9): Xaa can be S, P, or A
  misc_feature (11)..(11): Xaa can be L, H, or F
  misc_feature (13)..(13): Xaa can be D or N
SDIFXGEPXLXPX

SEQ ID NO: 46 - protein, 13 aa, Artificial sequence
  IL-23p19 fragment
  misc_feature (4)..(4): Xaa can be T or K
  misc_feature (8)..(8): Xaa can be S, P, or A
  misc_feature (10)..(10): Xaa can be L, H, or F
  misc_feature (12)..(12): Xaa can be D or N
  misc_feature (13)..(13): Xaa can be G, S, or D
DIFXGEPXLXPXX

SEQ ID NO: 47 - protein, 13 aa, Artificial sequence
  IL-23p19 fragment
  misc_feature (3)..(3): Xaa can be T or K
  misc_feature (7)..(7): Xaa can be S, P, or A
  misc_feature (9)..(9): Xaa can be L, H, or F
  misc_feature (11)..(11): Xaa can be D or N
  misc_feature (12)..(12): Xaa can be G, S, or D
  misc_feature (13)..(13): Xaa can be P or S
IFXGEPXLXPXXX

SEQ ID NO: 48 - protein, 13 aa, Artificial sequence
  IL-23p19 fragment
  misc_feature (2)..(2): Xaa can be T or K
  misc_feature (6)..(6): Xaa can be S, P, or A
  misc_feature (8)..(8): Xaa can be L, H, or F
  misc_feature (10)..(10): Xaa can be D or N
  misc_feature (11)..(11): Xaa can be G, S, or D
  misc_feature (12)..(12): Xaa can be P or S
  misc_feature (13)..(13): Xaa can be V or M
FXGEPXLXPXXXX

SEQ ID NO: 49 - protein, 13 aa, Artificial sequence
  IL-23p19 fragment
  misc_feature (1)..(1): Xaa can be T or K
  misc_feature (5)..(5): Xaa can be S, P, or A
  misc_feature (7)..(7): Xaa can be L, H, or F
  misc_feature (9)..(9): Xaa can be D or N
  misc_feature (10)..(10): Xaa can be G, S, or D
  misc_feature (11)..(11): Xaa can be P or S
  misc_feature (12)..(12): Xaa can be V or M
  misc_feature (13)..(13): Xaa can be G, D, S, E, or A
XGEPXLXPXXXXX

SEQ ID NO: 50 - protein, 13 aa, Artificial sequence
  IL-23p19 fragment
  misc_feature (4)..(4): Xaa can be S, P, or A
  misc_feature (6)..(6): Xaa can be L, H, or F
  misc_feature (8)..(8): Xaa can be D or N
  misc_feature (9)..(9): Xaa can be G, S, or D
  misc_feature (10)..(10): Xaa can be P or S
  misc_feature (11)..(11): Xaa can be V or M
  misc_feature (12)..(12): Xaa can be G, D, S, E, or A
GEPXLXPXXXXXQ

SEQ ID NO: 51 - protein, 13 aa, Artificial sequence
  IL-23p19 fragment
  misc_feature (3)..(3): Xaa can be S, P, or A
  misc_feature (5)..(5): Xaa can be L, H, or F
  misc_feature (7)..(7): Xaa can be D or N
  misc_feature (8)..(8): Xaa can be G, S, or D
  misc_feature (9)..(9): Xaa can be P or S
  misc_feature (10)..(10): Xaa can be V or M
  misc_feature (11)..(11): Xaa can be G, D, S, E, or A
EPXLXPXXXXXQL

SEQ ID NO: 52 - protein, 14 aa, Artificial sequence
  IL-23p19 fragment
  misc_feature (1)..(1): Xaa can be G, D, or A
  misc_feature (6)..(6): Xaa can be T or K
  misc_feature (10)..(10): Xaa can be S, P, or A
  misc_feature (12)..(12): Xaa can be L, H, or F
  misc_feature (14)..(14): Xaa can be D or N
XSDIFXGEPXLXPX

SEQ ID NO: 53 - protein, 14 aa, Artificial sequence
  IL-23p19 fragment
  misc_feature (5)..(5): Xaa can be T or K
  misc_feature (9)..(9): Xaa can be S, P, or A
  misc_feature (11)..(11): Xaa can be L, H, or F
  misc_feature (13)..(13): Xaa can be D or N
  misc_feature (14)..(14): Xaa can be G, S, or D
SDIFXGEPXLXPXX

SEQ ID NO: 54 - protein, 14 aa, Artificial sequence
  IL-23p19 fragment
  misc_feature (4)..(4): Xaa can be T or K
  misc_feature (8)..(8): Xaa can be S, P, or A
  misc_feature (10)..(10): Xaa can be L, H, or F
  misc_feature (12)..(12): Xaa can be D or N
  misc_feature (13)..(13): Xaa can be G, S, or D
  misc_feature (14)..(14): Xaa can be P or S
DIFXGEPXLXPXXX

SEQ ID NO: 55 - protein, 14 aa, Artificial sequence
  IL-23p19 fragment
  misc_feature (3)..(3): Xaa can be T or K
  misc_feature (7)..(7): Xaa can be S, P, or A
  misc_feature (9)..(9): Xaa can be L, H, or F
  misc_feature (11)..(11): Xaa can be D or N
  misc_feature (12)..(12): Xaa can be G, S, or D
  misc_feature (13)..(13): Xaa can be P or S
  misc_feature (14)..(14): Xaa can be V or M
IFXGEPXLXPXXXX

SEQ ID NO: 56 - protein, 14 aa, Artificial sequence
  IL-23p19 fragment
  misc_feature (2)..(2): Xaa can be T or K
  misc_feature (6)..(6): Xaa can be S, P, or A
  misc_feature (8)..(8): Xaa can be L, H, or F
  misc_feature (10)..(10): Xaa can be D or N
  misc_feature (11)..(11): Xaa can be G, S, or D
  misc_feature (12)..(12): Xaa can be P or S
  misc_feature (13)..(13): Xaa can be V or M
  misc_feature (14)..(14): Xaa can be G, D, S, E, or A
FXGEPXLXPXXXXX

SEQ ID NO: 57 - protein, 14 aa, Artificial sequence
  IL-23p19 fragment
  misc_feature (1)..(1): Xaa can be T or K
  misc_feature (5)..(5): Xaa can be S, P, or A
  misc_feature (7)..(7): Xaa can be L, H, or F
  misc_feature (9)..(9): Xaa can be D or N
  misc_feature (10)..(10): Xaa can be G, S, or D
  misc_feature (11)..(11): Xaa can be P or S
  misc_feature (12)..(12): Xaa can be V or M
  misc_feature (13)..(13): Xaa can be G, D, S, E, or A
XGEPXLXPXXXXXQ

SEQ ID NO: 58 - protein, 14 aa, Artificial sequence
  IL-23p19 fragment
  misc_feature (4)..(4): Xaa can be S, P, or A
  misc_feature (6)..(6): Xaa can be L, H, or F
  misc_feature (8)..(8): Xaa can be D or N
  misc_feature (9)..(9): Xaa can be G, S, or D
  misc_feature (10)..(10): Xaa can be P or S
  misc_feature (11)..(11): Xaa can be V or M
  misc_feature (12)..(12): Xaa can be G, D, S, E, or A
GEPXLXPXXXXXQL

SEQ ID NO: 59 - protein, 15 aa, Artificial sequence
  IL-23p19 fragment
  misc_feature (1)..(1): Xaa can be G, D, or A
  misc_feature (6)..(6): Xaa can be T or K
  misc_feature (10)..(10): Xaa can be S, P, or A
  misc_feature (12)..(12): Xaa can be L, H, or F
  misc_feature (14)..(14): Xaa can be D or N
  misc_feature (15)..(15): Xaa can be G, S, or D
XSDIFXGEPXLXPXX

SEQ ID NO: 60 - protein, 15 aa, Artificial sequence
  IL-23p19 fragment
  misc_feature (5)..(5): Xaa can be T or K
  misc_feature (9)..(9): Xaa can be S, P, or A
  misc_feature (11)..(11): Xaa can be L, H, or F
  misc_feature (13)..(13): Xaa can be D or N
  misc_feature (14)..(14): Xaa can be G, S, or D
  misc_feature (15)..(15): Xaa can be P or S
SDIFXGEPXLXPXXX

SEQ ID NO: 61 - protein, 15 aa, Artificial sequence
  IL-23p19 fragment
  misc_feature (4)..(4): Xaa can be T or K
  misc_feature (8)..(8): Xaa can be S, P, or A
  misc_feature (10)..(10): Xaa can be L, H, or F
  misc_feature (12)..(12): Xaa can be D or N
  misc_feature (13)..(13): Xaa can be G, S, or D
  misc_feature (14)..(14): Xaa can be P or S
  misc_feature (15)..(15): Xaa can be V or M
DIFXGEPXLXPXXXX

SEQ ID NO: 62 - protein, 15 aa, Artificial sequence
  IL-23p19 fragment
  misc_feature (3)..(3): Xaa can be T or K
  misc_feature (7)..(7): Xaa can be S, P, or A
  misc_feature (9)..(9): Xaa can be L, H, or F
  misc_feature (11)..(11): Xaa can be D or N
  misc_feature (12)..(12): Xaa can be G, S, or D
  misc_feature (13)..(13): Xaa can be P or S
  misc_feature (14)..(14): Xaa can be V or M
  misc_feature (15)..(15): Xaa can be G, D, S, E, or A
IFXGEPXLXPXXXXX

SEQ ID NO: 63 - protein, 15 aa, Artificial sequence
  IL-23p19 fragment
  misc_feature (2)..(2): Xaa can be T or K
  misc_feature (6)..(6): Xaa can be S, P, or A
  misc_feature (8)..(8): Xaa can be L, H, or F
  misc_feature (10)..(10): Xaa can be D or N
  misc_feature (11)..(11): Xaa can be G, S, or D
  misc_feature (12)..(12): Xaa can be P or S
  misc_feature (13)..(13): Xaa can be V or M
  misc_feature (14)..(14): Xaa can be G, D, S, E, or A
FXGEPXLXPXXXXXQ

SEQ ID NO: 64 - protein, 15 aa, Artificial sequence
  IL-23p19 fragment
  misc_feature (1)..(1): Xaa can be T or K
  misc_feature (5)..(5): Xaa can be S, P, or A
  misc_feature (7)..(7): Xaa can be L, H, or F
  misc_feature (9)..(9): Xaa can be D or N
  misc_feature (10)..(10): Xaa can be G, S, or D
  misc_feature (11)..(11): Xaa can be P or S
  misc_feature (12)..(12): Xaa can be V or M
  misc_feature (13)..(13): Xaa can be G, D, S, E, or A
XGEPXLXPXXXXXQL

SEQ ID NO: 65 - protein, 16 aa, Artificial sequence
  IL-23p19 fragment
  misc_feature (1)..(1): Xaa can be G, D, or A
  misc_feature (6)..(6): Xaa can be T or K
  misc_feature (10)..(10): Xaa can be S, P, or A
  misc_feature (12)..(12): Xaa can be L, H, or F
  misc_feature (14)..(14): Xaa can be D or N
  misc_feature (15)..(15): Xaa can be G, S, or D
  misc_feature (16)..(16): Xaa can be P or S
XSDIFXGEPXLXPXXX

SEQ ID NO: 66 - protein, 16 aa, Artificial sequence
  IL-23p19 fragment
  misc_feature (5)..(5): Xaa can be T or K
  misc_feature (9)..(9): Xaa can be S, P, or A
  misc_feature (11)..(11): Xaa can be L, H, or F
  misc_feature (13)..(13): Xaa can be D or N
  misc_feature (14)..(14): Xaa can be G, S, or D
  misc_feature (15)..(15): Xaa can be P or S
  misc_feature (16)..(16): Xaa can be V or M
SDIFXGEPXLXPXXXX

SEQ ID NO: 67 - protein, 16 aa, Artificial sequence
  IL-23p19 fragment
  misc_feature (4)..(4): Xaa can be T or K
  misc_feature (8)..(8): Xaa can be S, P, or A
  misc_feature (10)..(10): Xaa can be L, H, or F
  misc_feature (12)..(12): Xaa can be D or N
  misc_feature (13)..(13): Xaa can be G, S, or D
  misc_feature (14)..(14): Xaa can be P or S
  misc_feature (15)..(15): Xaa can be V or M
  misc_feature (16)..(16): Xaa can be G, D, S, E, or A
DIFXGEPXLXPXXXXX

SEQ ID NO: 68 - protein, 16 aa, Artificial sequence
  IL-23p19 fragment
  misc_feature (3)..(3): Xaa can be T or K
  misc_feature (7)..(7): Xaa can be S, P, or A
  misc_feature (9)..(9): Xaa can be L, H, or F
  misc_feature (11)..(11): Xaa can be D or N
  misc_feature (12)..(12): Xaa can be G, S, or D
  misc_feature (13)..(13): Xaa can be P or S
  misc_feature (14)..(14): Xaa can be V or M
  misc_feature (15)..(15): Xaa can be G, D, S, E, or A
IFXGEPXLXPXXXXXQ

SEQ ID NO: 69 - protein, 16 aa, Artificial sequence
  IL-23p19 fragment
  misc_feature (2)..(2): Xaa can be T or K
  misc_feature (6)..(6): Xaa can be S, P, or A
  misc_feature (8)..(8): Xaa can be L, H, or F
  misc_feature (10)..(10): Xaa can be D or N
  misc_feature (11)..(11): Xaa can be G, S, or D
  misc_feature (12)..(12): Xaa can be P or S
  misc_feature (13)..(13): Xaa can be V or M
  misc_feature (14)..(14): Xaa can be G, D, S, E, or A
FXGEPXLXPXXXXXQL

SEQ ID NO: 70 - protein, 17 aa, Artificial sequence
  IL-23p19 fragment
  misc_feature (1)..(1): Xaa can be G, D, or A
  misc_feature (6)..(6): Xaa can be T or K
  misc_feature (10)..(10): Xaa can be S, P, or A
  misc_feature (12)..(12): Xaa can be L, H, or F
  misc_feature (14)..(14): Xaa can be D or N
  misc_feature (15)..(15): Xaa can be G, S, or D
  misc_feature (16)..(16): Xaa can be P or S
  misc_feature (17)..(17): Xaa can be V or M
XSDIFXGEPXLXPXXXX

SEQ ID NO: 71 - protein, 17 aa, Artificial sequence
  IL-23p19 fragment
  misc_feature (5)..(5): Xaa can be T or K
  misc_feature (9)..(9): Xaa can be S, P, or A
  misc_feature (11)..(11): Xaa can be L, H, or F
  misc_feature (13)..(13): Xaa can be D or N
  misc_feature (14)..(14): Xaa can be G, S, or D
  misc_feature (15)..(15): Xaa can be P or S
  misc_feature (16)..(16): Xaa can be V or M
  misc_feature (17)..(17): Xaa can be G, D, S, E, or A
SDIFXGEPXLXPXXXXX

SEQ ID NO: 72 - protein, 17 aa, Artificial sequence
  IL-23p19 fragment
  misc_feature (4)..(4): Xaa can be T or K
  misc_feature (8)..(8): Xaa can be S, P, or A
  misc_feature (10)..(10): Xaa can be L, H, or F
  misc_feature (12)..(12): Xaa can be D or N
  misc_feature (13)..(13): Xaa can be G, S, or D
  misc_feature (14)..(14): Xaa can be P or S
  misc_feature (15)..(15): Xaa can be V or M
  misc_feature (16)..(16): Xaa can be G, D, S, E, or A
DIFXGEPXLXPXXXXXQ

SEQ ID NO: 73 - protein, 17 aa, Artificial sequence
  IL-23p19 fragment
  misc_feature (3)..(3): Xaa can be T or K
  misc_feature (7)..(7): Xaa can be S, P, or A
  misc_feature (9)..(9): Xaa can be L, H, or F
  misc_feature (11)..(11): Xaa can be D or N
  misc_feature (12)..(12): Xaa can be G, S, or D
  misc_feature (13)..(13): Xaa can be P or S
  misc_feature (14)..(14): Xaa can be V or M
  misc_feature (15)..(15): Xaa can be G, D, S, E, or A
IFXGEPXLXPXXXXXQL

SEQ ID NO: 74 - protein, 18 aa, Artificial sequence
  IL-23p19 fragment
  misc_feature (1)..(1): Xaa can be G, D, or A
  misc_feature (6)..(6): Xaa can be T or K
  misc_feature (10)..(10): Xaa can be S, P, or A
  misc_feature (12)..(12): Xaa can be L, H, or F
  misc_feature (14)..(14): Xaa can be D or N
  misc_feature (15)..(15): Xaa can be G, S, or D
  misc_feature (16)..(16): Xaa can be P or S
  misc_feature (17)..(17): Xaa can be V or M
  misc_feature (18)..(18): Xaa can be G, D, S, E, or A
XSDIFXGEPXLXPXXXXX

SEQ ID NO: 75 - protein, 18 aa, Artificial sequence
  IL-23p19 fragment
  misc_feature (5)..(5): Xaa can be T or K
  misc_feature (9)..(9): Xaa can be S, P, or A
  misc_feature (11)..(11): Xaa can be L, H, or F
  misc_feature (13)..(13): Xaa can be D or N
  misc_feature (14)..(14): Xaa can be G, S, or D
  misc_feature (15)..(15): Xaa can be P or S
  misc_feature (16)..(16): Xaa can be V or M
  misc_feature (17)..(17): Xaa can be G, D, S, E, or A
SDIFXGEPXLXPXXXXXQ

SEQ ID NO: 76 - protein, 18 aa, Artificial sequence
  IL-23p19 fragment
  misc_feature (4)..(4): Xaa can be T or K
  misc_feature (8)..(8): Xaa can be S, P, or A
  misc_feature (10)..(10): Xaa can be L, H, or F
  misc_feature (12)..(12): Xaa can be D or N
  misc_feature (13)..(13): Xaa can be G, S, or D
  misc_feature (14)..(14): Xaa can be P or S
  misc_feature (15)..(15): Xaa can be V or M
  misc_feature (16)..(16): Xaa can be G, D, S, E, or A
DIFXGEPXLXPXXXXXQL

SEQ ID NO: 77 - protein, 19 aa, Artificial sequence
  IL-23p19 fragment
  misc_feature (1)..(1): Xaa can be G, D, or A
  misc_feature (6)..(6): Xaa can be T or K
  misc_feature (10)..(10): Xaa can be S, P, or A
  misc_feature (12)..(12): Xaa can be L, H, or F
  misc_feature (14)..(14): Xaa can be D or N
  misc_feature (15)..(15): Xaa can be G, S, or D
  misc_feature (16)..(16): Xaa can be P or S
  misc_feature (17)..(17): Xaa can be V or M
  misc_feature (18)..(18): Xaa can be G, D, S, E, or A
XSDIFXGEPXLXPXXXXXQ

SEQ ID NO: 78 - protein, 19 aa, Artificial sequence
  IL-23p19 fragment
  misc_feature (5)..(5): Xaa can be T or K
  misc_feature (9)..(9): Xaa can be S, P, or A
  misc_feature (11)..(11): Xaa can be L, H, or F
  misc_feature (13)..(13): Xaa can be D or N
  misc_feature (14)..(14): Xaa can be G, S, or D
  misc_feature (15)..(15): Xaa can be P or S
  misc_feature (16)..(16): Xaa can be V or M
  misc_feature (17)..(17): Xaa can be G, D, S, E, or A
SDIFXGEPXLXPXXXXXQL

SEQ ID NO: 79 - protein, 20 aa, Artificial sequence
  IL-23p19 fragment
  misc_feature (1)..(1): Xaa can be G, D, or A
  misc_feature (6)..(6): Xaa can be T or K
  misc_feature (10)..(10): Xaa can be S, P, or A
  misc_feature (12)..(12): Xaa can be L, H, or F
  misc_feature (14)..(14): Xaa can be D or N
  misc_feature (15)..(15): Xaa can be G, S, or D
  misc_feature (16)..(16): Xaa can be P or S
  misc_feature (17)..(17): Xaa can be V or M
  misc_feature (18)..(18): Xaa can be G, D, S, E, or A
XSDIFXGEPXLXPXXXXXQL

SEQ ID NO: 80 - protein, 11 aa, Artificial sequence
  IL-23p19 fragment
GSDIFTGEPSL

SEQ ID NO: 81 - protein, 11 aa, Artificial sequence
  IL-23p19 fragment
SDIFTGEPSLL

SEQ ID NO: 82 - protein, 11 aa, Artificial sequence
  IL-23p19 fragment
DIFTGEPSLLP

SEQ ID NO: 83 - protein, 11 aa, Artificial sequence
  IL-23p19 fragment
IFTGEPSLLPD

SEQ ID NO: 84 - protein, 11 aa, Artificial sequence
  IL-23p19 fragment
FTGEPSLLPDS

SEQ ID NO: 85 - protein, 11 aa, Artificial sequence
  IL-23p19 fragment
TGEPSLLPDSP

SEQ ID NO: 86 - protein, 11 aa, Artificial sequence
  IL-23p19 fragment
KGEPSLLPDSP

SEQ ID NO: 87 - protein, 11 aa, Artificial sequence
  IL-23p19 fragment
GEPSLLPDSPV

SEQ ID NO: 88 - protein, 11 aa, Artificial sequence
  IL-23p19 fragment
EPSLLPDSPVG

SEQ ID NO: 89 - protein, 11 aa, Artificial sequence
  IL-23p19 fragment
PSLLPDSPVGQ

SEQ ID NO: 90 - protein, 11 aa, Artificial sequence
  IL-23p19 fragment
SLLPDSPVGQL

SEQ ID NO: 91 - protein, 12 aa, Artificial sequence
  IL-23p19 fragment
GSDIFTGEPSLL

SEQ ID NO: 92 - protein, 12 aa, Artificial sequence
  IL-23p19 fragment
SDIFTGEPSLLP

SEQ ID NO: 93 - protein, 12 aa, Artificial sequence
  IL-23p19 fragment
DIFTGEPSLLPD

SEQ ID NO: 94 - protein, 12 aa, Artificial sequence
  IL-23p19 fragment
IFTGEPSLLPDS

SEQ ID NO: 95 - protein, 12 aa, Artificial sequence
  IL-23p19 fragment
FTGEPSLLPDSP

SEQ ID NO: 96 - protein, 12 aa, Artificial sequence
  IL-23p19 fragment
TGEPSLLPDSPV

SEQ ID NO: 97 - protein, 12 aa, Artificial sequence
  IL-23p19 fragment
GEPSLLPDSPVG

SEQ ID NO: 98 - protein, 12 aa, Artificial sequence
  IL-23p19 fragment
EPSLLPDSPVGQ

SEQ ID NO: 99 - protein, 12 aa, Artificial sequence
  IL-23p19 fragment
PSLLPDSPVGQL

SEQ ID NO: 100 - protein, 13 aa, Artificial sequence
  IL-23p19 fragment
GSDIFTGEPSLLP

SEQ ID NO: 101 - protein, 13 aa, Artificial sequence
  IL-23p19 fragment
SDIFTGEPSLLPD

SEQ ID NO: 102 - protein, 13 aa, Artificial sequence
  IL-23p19 fragment
DIFTGEPSLLPDS

SEQ ID NO: 103 - protein, 13 aa, Artificial sequence
  IL-23p19 fragment
IFTGEPSLLPDSP

SEQ ID NO: 104 - protein, 13 aa, Artificial sequence
  IL-23p19 fragment
FTGEPSLLPDSPV

SEQ ID NO: 105 - protein, 13 aa, Artificial sequence
  IL-23p19 fragment
TGEPSLLPDSPVG

SEQ ID NO: 106 - protein, 13 aa, Artificial sequence
  IL-23p19 fragment
GEPSLLPDSPVGQ

SEQ ID NO: 107 - protein, 13 aa, Artificial sequence
  IL-23p19 fragment
EPSLLPDSPVGQL

SEQ ID NO: 108 - protein, 14 aa, Artificial sequence
  IL-23p19
GSDIFTGEPSLLPD

SEQ ID NO: 109 - protein, 14 aa, Artificial sequence
  IL-23p19 fragment
SDIFTGEPSLLPDS

SEQ ID NO: 110 - protein, 14 aa, Artificial sequence
  IL-23p19 fragment
DIFTGEPSLLPDSP

SEQ ID NO: 111 - protein, 14 aa, Artificial sequence
  IL-23p19 fragment
IFTGEPSLLPDSPV

SEQ ID NO: 112 - protein, 14 aa, Artificial sequence
  IL-23p19 fragment
FTGEPSLLPDSPVG

SEQ ID NO: 113 - protein, 14 aa, Artificial sequence
  IL-23p19 fragment
TGEPSLLPDSPVGQ

SEQ ID NO: 114 - protein, 14 aa, Artificial sequence
  IL-23p19 fragment
GEPSLLPDSPVGQL

SEQ ID NO: 115 - protein, 15 aa, Artificial sequence
  IL-23p19 fragment
GSDIFTGEPSLLPDS

SEQ ID NO: 116 - protein, 15 aa, Artificial sequence
  IL-23p19 fragment
SDIFTGEPSLLPDSP

SEQ ID NO: 117 - protein, 15 aa, Artificial sequence
  IL-23p19 fragment
DIFTGEPSLLPDSPV

SEQ ID NO: 118 - protein, 15 aa, Artificial sequence
  IL-23p19 fragment
IFTGEPSLLPDSPVG

SEQ ID NO: 119 - protein, 15 aa, Artificial sequence
  IL-23p19 fragment
FTGEPSLLPDSPVGQ

SEQ ID NO: 120 - protein, 15 aa, Artificial sequence
  IL-23p19
TGEPSLLPDSPVGQL

SEQ ID NO: 121 - protein, 16 aa, Artificial sequence
  IL-23p19 fragment
GSDIFTGEPSLLPDSP

SEQ ID NO: 122 - protein, 16 aa, Artificial sequence
  IL-23p19 fragment
SDIFTGEPSLLPDSPV

SEQ ID NO: 123 - protein, 16 aa, Artificial sequence
  IL-23p19 fragment
DIFTGEPSLLPDSPVG

SEQ ID NO: 124 - protein, 16 aa, Artificial sequence
  IL-23p19 fragment
IFTGEPSLLPDSPVGQ

SEQ ID NO: 125 - protein, 16 aa, Artificial sequence
  IL-23p19 fragment
FTGEPSLLPDSPVGQL

SEQ ID NO: 126 - protein, 17 aa, Artificial sequence
  IL-23p19 fragment
GSDIFTGEPSLLPDSPV

SEQ ID NO: 127 - protein, 17 aa, Artificial sequence
  IL-23p19 fragment
SDIFTGEPSLLPDSPVG

SEQ ID NO: 128 - protein, 17 aa, Artificial sequence
  IL-23p19 fragment
DIFTGEPSLLPDSPVGQ

SEQ ID NO: 129 - protein, 17 aa, Artificial sequence
  IL-23p19 fragment
IFTGEPSLLPDSPVGQL

SEQ ID NO: 130 - protein, 18 aa, Artificial sequence
  IL-23p19 fragment
GSDIFTGEPSLLPDSPVG

SEQ ID NO: 131 - protein, 18 aa, Artificial sequence
  IL-23p19 fragment
SDIFTGEPSLLPDSPVGQ

SEQ ID NO: 132 - protein, 18 aa, Artificial sequence
  IL-23p19 fragment
DIFTGEPSLLPDSPVGQL

SEQ ID NO: 133 - protein, 19 aa, Artificial sequence
  IL-23p19 fragment
GSDIFTGEPSLLPDSPVGQ

SEQ ID NO: 134 - protein, 19 aa, Artificial sequence
  IL-23p19 fragment
SDIFTGEPSLLPDSPVGQL

SEQ ID NO: 135 - protein, 20 aa, Artificial sequence
  IL-23p19 fragment
ASDIFTGEPSLLPDSPVAQL

SEQ ID NO: 136 - protein, 20 aa, Artificial sequence
  IL-23p19 fragment
ASDIFTGEPSLLPDSPVGQL

SEQ ID NO: 137 - protein, 20 aa, Artificial sequence
  IL-23p19 fragment
GSDIFTGEPSLLPDSPVAQL

SEQ ID NO: 138 - protein, 20 aa, Artificial sequence
  IL-23p19 fragment
DSDIFTGEPALLPDSPVEQL

SEQ ID NO: 139 - protein, 21 aa, Artificial sequence
  IL-23p19 fragment
YEKLLGSDICTGEPSLLPDSP

SEQ ID NO: 140 - protein, 25 aa, Artificial sequence
  IL-23p19 fragment
YEKLCGSDIFTGEPSLLPDSPVGQL

SEQ ID NO: 141 - protein, 26 aa, Artificial sequence
  IL-23p19 fragment
KLLGSDIFTGEPSLLPDSPVGQLHAS